European Patent Specification EP 3 778 781 B1, published July 1, 2026. Title: A molded article and a method for producing the same. Applicant: Spiber Inc. The sequence listing filed with the application follows.

SEQUENCE LISTING (40 sequences)

SEQ ID NO: 1 - protein, 50 aa, Araneus diadematus
SGCDVLVQALLEVVSALVSILGSSSIGQINYGASAQYTQMVGQSVAQALA

SEQ ID NO: 2 - protein, 30 aa, Araneus diadematus
SGCDVLVQALLEVVSALVSILGSSSIGQIN

SEQ ID NO: 3 - protein, 21 aa, Araneus diadematus
SGCDVLVQALLEVVSALVSIL

SEQ ID NO: 4 - protein, 1154 aa, Artificial Sequence
  recombinant spider silk protein ADF3KaiLargeNRSH1
MHHHHHHHHHHSSGSSLEVLFQGPARAGSGQQGPGQQGPGQQGPGQQGPYGPGASAAAAAAGGYGPGSGQQGPSQQGPGQQGPGGQGPYGPGASAAAAAAGGYGPGSGQQGPGGQGPYGPGSSAAAAAAGGNGPGSGQQGAGQQGPGQQGPGASAAAAAAGGYGPGSGQQGPGQQGPGGQGPYGPGASAAAAAAGGYGPGSGQGPGQQGPGGQGPYGPGASAAAAAAGGYGPGSGQQGPGQQGPGQQGPGGQGPYGPGASAAAAAAGGYGPGYGQQGPGQQGPGGQGPYGPGASAASAASGGYGPGSGQQGPGQQGPGGQGPYGPGASAAAAAAGGYGPGSGQQGPGQQGPGQQGPGQQGPGGQGPYGPGASAAAAAAGGYGPGSGQQGPGQQGPGQQGPGQQGPGQQGPGQQGPGQQGPGQQGPGQQGPGGQGAYGPGASAAAGAAGGYGPGSGQQGPGQQGPGQQGPGQQGPGQQGPGQQGPGQQGPGQQGPYGPGASAAAAAAGGYGPGSGQQGPGQQGPGQQGPGGQGPYGPGAASAAVSVSRARAGSGQQGPGQQGPGQQGPGQQGPYGPGASAAAAAAGGYGPGSGQQGPSQQGPGQQGPGGQGPYGPGASAAAAAAGGYGPGSGQQGPGGQGPYGPGSSAAAAAAGGNGPGSGQQGAGQQGPGQQGPGASAAAAAAGGYGPGSGQQGPGQQGPGGQGPYGPGASAAAAAAGGYGPGSGQGPGQQGPGGQGPYGPGASAAAAAAGGYGPGSGQQGPGQQGPGQQGPGGQGPYGPGASAAAAAAGGYGPGYGQQGPGQQGPGGQGPYGPGASAASAASGGYGPGSGQQGPGQQGPGGQGPYGPGASAAAAAAGGYGPGSGQQGPGQQGPGQQGPGQQGPGGQGPYGPGASAAAAAAGGYGPGSGQQGPGQQGPGQQGPGQQGPGQQGPGQQGPGQQGPGQQGPGQQGPGGQGAYGPGASAAAGAAGGYGPGSGQQGPGQQGPGQQGPGQQGPGQQGPGQQGPGQQGPGQQGPYGPGASAAAAAAGGYGPGSGQQGPGQQGPGQQGPGGQGPYGPGAASAAVSVGGYGPQSSSVPVASAVASRLSSPAASSRVSSAVSSLVSSGPTKHAALSNTISSVVSQVSASNPGLSGCDVLVQALLEVVSALVSIL

SEQ ID NO: 5 - protein, 24 aa, Artificial Sequence
  His tag and start codon
MHHHHHHHHHHSSGSSLEVLFQGP

SEQ ID NO: 6 - protein, 597 aa, Artificial Sequence
  Met-PRT380
MGPGQQGPYGPGASAAAAAGQNGPGSGQQGPGQSAAAAAGQYGPGQQGPGQQGPGSSAAAAAGPGQYGPGQQGPSASAAAAAGPGSGQQGPGASAAAAAGQYGPGQQGPGQQGPGSSAAAAAGQYGSGPGQQGPYGSAAAAAGPGSGQYGQGPYGPGASAAAAAGPGQYGPGQQGPSASAAAAAGSGQQGPGQYGPYASAAAAAGQYGSGPGQQGPYGPGQSAAAAAGSGQQGPGQQGPYASAAAAAGPGQQGPYGPGSSAAAAAGQYGYGPGQQGPYGPGASAAAAAGQNGPGSGQYGPGQQGPGQSAAAAAGPGQQGPYGPGASAAAAAGQYGPGQQGPGQYGPGSSAAAAAGPGQQGPYGPGSSAAAAAGQYGPGQQGPYGPGQSAAAAAGQYQQGPGQQGPYGPGASAAAAAGPGQQGPYGPGASAAAAAGPGQYGPGQQGPSASAAAAAGQYGSGPGQYGPYGPGQSAAAAAGPGSGQQGQGPYGPGASAAAAAGQYGPGQQGPYGPGQSAAAAAGPGSGQYGPGASAAAAAGQNGPGSGQYGPGQQGPGQSAAAAAGQYQQGPGQQGPYGPGASAAAAAGPGSGQQGPGAS

SEQ ID NO: 7 - protein, 590 aa, Artificial Sequence
  Met-PRT410
MGPGQQGPYGPGASAAAAAGQNGPGSGQQGPGQSGQYGPGQQGPGQQGPGSSAAAAAGPGQYGPGQQGPSASAAAAAGPGSGQQGPGASGQYGPGQQGPGQQGPGSSAAAAAGQYGSGPGQQGPYGSAAAAAGPGSGQYGQGPYGPGASGPGQYGPGQQGPSASAAAAAGSGQQGPGQYGPYASAAAAAGQYGSGPGQQGPYGPGQSGSGQQGPGQQGPYASAAAAAGPGQQGPYGPGSSAAAAAGQYGYGPGQQGPYGPGASGQNGPGSGQYGPGQQGPGQSAAAAAGPGQQGPYGPGASAAAAAGQYGPGQQGPGQYGPGSSGPGQQGPYGPGSSAAAAAGQYGPGQQGPYGPGQSAAAAAGQYQQGPGQQGPYGPGASGPGQQGPYGPGASAAAAAGPGQYGPGQQGPSASAAAAAGQYGSGPGQYGPYGPGQSGPGSGQQGQGPYGPGASAAAAAGQYGPGQQGPYGPGQSAAAAAGPGSGQYGPGASGQNGPGSGQYGPGQQGPGQSAAAAAGQYQQGPGQQGPYGPGASAAAAAGQYGSGPGQQGPYGPGQSGSGQQGPGQQGPYASAAAAAGPGSGQQGPGAS

SEQ ID NO: 8 - protein, 565 aa, Artificial Sequence
  Met-PRT468
MGPGQQGPYGPGASAAAAAAAGSNGPGSGQQGPGQSGQYGPGQQGPGQQGPGSSAAAAAAAGPGQYGPGQQGPSASAAAAAAAGPGSGQQGPGASGQYGPGQQGPGQQGPGSSAAAAAAAGSYGSGPGQQGPYGSAAAAAAAGPGSGQYGQGPYGPGASGPGQYGPGQQGPSASAAAAAAAGSGQQGPGQYGPYASAAAAAAAGSYGSGPGQQGPYGPGQSGSGQQGPGQQGPYASAAAAAAAGPGQQGPYGPGSSAAAAAAAGSYGYGPGQQGPYGPGASGQNGPGSGQYGPGQQGPGPSAAAAAAAGPGQQGPYGPGASAAAAAAAGSYGPGQQGPGQYGPGSSGPGQQGPYGPGSSAAAAAAAGSYGPGQQGPYGPGPSAAAAAAAGSYQQGPGQQGPYGPGASGPGQQGPYGPGASAAAAAAAGPGQYGPGQQGPSASAAAAAAAGSYGSGPGQYGPYGPGQSGPGSGQQGQGPYGPGASAAAAAAAGSYGPGQQGPYGPGPSAAAAAAAGPGSGQYGPGASGQNGPGSGQYGPGQQGPGPSAAAAAAAGPGSGQQGPGAS

SEQ ID NO: 9 - protein, 2364 aa, Artificial Sequence
  Met-PRT799
MGPGQQGPYGPGASAAAAAGQNGPGSGQQGPGQSGQYGPGQQGPGQQGPGSSAAAAAGPGQYGPGQQGPSASAAAAAGPGSGQQGPGASGQYGPGQQGPGQQGPGSSAAAAAGQYGSGPGQQGPYGSAAAAAGPGSGQYGQGPYGPGASGPGQYGPGQQGPSASAAAAAGSGQQGPGQYGPYASAAAAAGQYGSGPGQQGPYGPGQSGSGQQGPGQQGPYASAAAAAGPGQQGPYGPGSSAAAAAGQYGYGPGQQGPYGPGASGQNGPGSGQYGPGQQGPGQSAAAAAGPGQQGPYGPGASAAAAAGQYGPGQQGPGQYGPGSSGPGQQGPYGPGSSAAAAAGQYGPGQQGPYGPGQSAAAAAGQYQQGPGQQGPYGPGASGPGQQGPYGPGASAAAAAGPGQYGPGQQGPSASAAAAAGQYGSGPGQYGPYGPGQSGPGSGQQGQGPYGPGASAAAAAGQYGPGQQGPYGPGQSAAAAAGPGSGQYGPGASGQNGPGSGQYGPGQQGPGQSAAAAAGQYQQGPGQQGPYGPGASAAAAAGQYGSGPGQQGPYGPGQSGSGQQGPGQQGPYASAAAAAGPGSGQQGPGASGQQGPYGPGASAAAAAGQNGPGSGQQGPGQSGQYGPGQQGPGQQGPGSSAAAAAGPGQYGPGQQGPSASAAAAAGPGSGQQGPGASGQYGPGQQGPGQQGPGSSAAAAAGQYGSGPGQQGPYGSAAAAAGPGSGQYGQGPYGPGASGPGQYGPGQQGPSASAAAAAGSGQQGPGQYGPYASAAAAAGQYGSGPGQQGPYGPGQSGSGQQGPGQQGPYASAAAAAGPGQQGPYGPGSSAAAAAGQYGYGPGQQGPYGPGASGQNGPGSGQYGPGQQGPGQSAAAAAGPGQQGPYGPGASAAAAAGQYGPGQQGPGQYGPGSSGPGQQGPYGPGSSAAAAAGQYGPGQQGPYGPGQSAAAAAGQYQQGPGQQGPYGPGASGPGQQGPYGPGASAAAAAGPGQYGPGQQGPSASAAAAAGQYGSGPGQYGPYGPGQSGPGSGQQGQGPYGPGASAAAAAGQYGPGQQGPYGPGQSAAAAAGPGSGQYGPGASGQNGPGSGQYGPGQQGPGQSAAAAAGQYQQGPGQQGPYGPGASAAAAAGQYGSGPGQQGPYGPGQSGSGQQGPGQQGPYASAAAAAGPGSGQQGPGASGQQGPYGPGASAAAAAGQNGPGSGQQGPGQSGQYGPGQQGPGQQGPGSSAAAAAGPGQYGPGQQGPSASAAAAAGPGSGQQGPGASGQYGPGQQGPGQQGPGSSAAAAAGQYGSGPGQQGPYGSAAAAAGPGSGQYGQGPYGPGASGPGQYGPGQQGPSASAAAAAGSGQQGPGQYGPYASAAAAAGQYGSGPGQQGPYGPGQSGSGQQGPGQQGPYASAAAAAGPGQQGPYGPGSSAAAAAGQYGYGPGQQGPYGPGASGQNGPGSGQYGPGQQGPGQSAAAAAGPGQQGPYGPGASAAAAAGQYGPGQQGPGQYGPGSSGPGQQGPYGPGSSAAAAAGQYGPGQQGPYGPGQSAAAAAGQYQQGPGQQGPYGPGASGPGQQGPYGPGASAAAAAGPGQYGPGQQGPSASAAAAAGQYGSGPGQYGPYGPGQSGPGSGQQGQGPYGPGASAAAAAGQYGPGQQGPYGPGQSAAAAAGPGSGQYGPGASGQNGPGSGQYGPGQQGPGQSAAAAAGQYQQGPGQQGPYGPGASAAAAAGQYGSGPGQQGPYGPGQSGSGQQGPGQQGPYASAAAAAGPGSGQQGPGASGQQGPYGPGASAAAAAGQNGPGSGQQGPGQSGQYGPGQQGPGQQGPGSSAAAAAGPGQYGPGQQGPSASAAAAAGPGSGQQGPGASGQYGPGQQGPGQQGPGSSAAAAAGQYGSGPGQQGPYGSAAAAAGPGSGQYGQGPYGPGASGPGQYGPGQQGPSASAAAAAGSGQQGPGQYGPYASAAAAAGQYGSGPGQQGPYGPGQSGSGQQGPGQQGPYASAAAAAGPGQQGPYGPGSSAAAAAGQYGYGPGQQGPYGPGASGQNGPGSGQYGPGQQGPGQSAAAAAGPGQQGPYGPGASAAAAAGQYGPGQQGPGQYGPGSSGPGQQGPYGPGSSAAAAAGQYGPGQQGPYGPGQSAAAAAGQYQQGPGQQGPYGPGASGPGQQGPYGPGASAAAAAGPGQYGPGQQGPSASAAAAAGQYGSGPGQYGPYGPGQSGPGSGQQGQGPYGPGASAAAAAGQYGPGQQGPYGPGQSAAAAAGPGSGQYGPGASGQNGPGSGQYGPGQQGPGQSAAAAAGQYQQGPGQQGPYGPGASAAAAAGQYGSGPGQQGPYGPGQSGSGQQGPGQQGPYASAAAAAGPGSGQQGSSVDKLAAALEHHHHHH

SEQ ID NO: 10 - protein, 597 aa, Artificial Sequence
  Met-PRT313
MGPGGQGPYGPGASAAAAAGGNGPGSGQQGPGGSAAAAAGGYGPGGQGPGQQGPGSSAAAAAGPGGYGPGGQGPSASAAAAAGPGSGQQGPGASAAAAAGGYGPGGQGPGQQGPGSSAAAAAGGYGSGPGQQGPYGSAAAAAGPGSGGYGQGPYGPGASAAAAAGPGGYGPGGQGPSASAAAAAGSGQQGPGGYGPYASAAAAAGGYGSGPGQQGPYGPGGSAAAAAGSGQQGPGQQGPYASAAAAAGPGGQGPYGPGSSAAAAAGGYGYGPGGQGPYGPGASAAAAAGGNGPGSGGYGPGQQGPGGSAAAAAGPGGQGPYGPGASAAAAAGGYGPGGQGPGGYGPGSSAAAAAGPGGQGPYGPGSSAAAAAGGYGPGQQGPYGPGGSAAAAAGGYQQGPGGQGPYGPGASAAAAAGPGGQGPYGPGASAAAAAGPGGYGPGGQGPSASAAAAAGGYGSGPGGYGPYGPGGSAAAAAGPGSGQQGQGPYGPGASAAAAAGGYGPGQQGPYGPGGSAAAAAGPGSGGYGPGASAAAAAGGNGPGSGGYGPGQQGPGGSAAAAAGGYQQGPGGQGPYGPGASAAAAAGPGSGQQGPGAS

SEQ ID NO: 11 - protein, 12 aa, Artificial Sequence
  HisTag
MHHHHHHSSGSS

SEQ ID NO: 12 - protein, 608 aa, Artificial Sequence
  PRT380
MHHHHHHSSGSSGPGQQGPYGPGASAAAAAGQNGPGSGQQGPGQSAAAAAGQYGPGQQGPGQQGPGSSAAAAAGPGQYGPGQQGPSASAAAAAGPGSGQQGPGASAAAAAGQYGPGQQGPGQQGPGSSAAAAAGQYGSGPGQQGPYGSAAAAAGPGSGQYGQGPYGPGASAAAAAGPGQYGPGQQGPSASAAAAAGSGQQGPGQYGPYASAAAAAGQYGSGPGQQGPYGPGQSAAAAAGSGQQGPGQQGPYASAAAAAGPGQQGPYGPGSSAAAAAGQYGYGPGQQGPYGPGASAAAAAGQNGPGSGQYGPGQQGPGQSAAAAAGPGQQGPYGPGASAAAAAGQYGPGQQGPGQYGPGSSAAAAAGPGQQGPYGPGSSAAAAAGQYGPGQQGPYGPGQSAAAAAGQYQQGPGQQGPYGPGASAAAAAGPGQQGPYGPGASAAAAAGPGQYGPGQQGPSASAAAAAGQYGSGPGQYGPYGPGQSAAAAAGPGSGQQGQGPYGPGASAAAAAGQYGPGQQGPYGPGQSAAAAAGPGSGQYGPGASAAAAAGQNGPGSGQYGPGQQGPGQSAAAAAGQYQQGPGQQGPYGPGASAAAAAGPGSGQQGPGAS

SEQ ID NO: 13 - protein, 601 aa, Artificial Sequence
  PRT410
MHHHHHHSSGSSGPGQQGPYGPGASAAAAAGQNGPGSGQQGPGQSGQYGPGQQGPGQQGPGSSAAAAAGPGQYGPGQQGPSASAAAAAGPGSGQQGPGASGQYGPGQQGPGQQGPGSSAAAAAGQYGSGPGQQGPYGSAAAAAGPGSGQYGQGPYGPGASGPGQYGPGQQGPSASAAAAAGSGQQGPGQYGPYASAAAAAGQYGSGPGQQGPYGPGQSGSGQQGPGQQGPYASAAAAAGPGQQGPYGPGSSAAAAAGQYGYGPGQQGPYGPGASGQNGPGSGQYGPGQQGPGQSAAAAAGPGQQGPYGPGASAAAAAGQYGPGQQGPGQYGPGSSGPGQQGPYGPGSSAAAAAGQYGPGQQGPYGPGQSAAAAAGQYQQGPGQQGPYGPGASGPGQQGPYGPGASAAAAAGPGQYGPGQQGPSASAAAAAGQYGSGPGQYGPYGPGQSGPGSGQQGQGPYGPGASAAAAAGQYGPGQQGPYGPGQSAAAAAGPGSGQYGPGASGQNGPGSGQYGPGQQGPGQSAAAAAGQYQQGPGQQGPYGPGASAAAAAGQYGSGPGQQGPYGPGQSGSGQQGPGQQGPYASAAAAAGPGSGQQGPGAS

SEQ ID NO: 14 - protein, 576 aa, Artificial Sequence
  PRT468
MHHHHHHSSGSSGPGQQGPYGPGASAAAAAAAGSNGPGSGQQGPGQSGQYGPGQQGPGQQGPGSSAAAAAAAGPGQYGPGQQGPSASAAAAAAAGPGSGQQGPGASGQYGPGQQGPGQQGPGSSAAAAAAAGSYGSGPGQQGPYGSAAAAAAAGPGSGQYGQGPYGPGASGPGQYGPGQQGPSASAAAAAAAGSGQQGPGQYGPYASAAAAAAAGSYGSGPGQQGPYGPGQSGSGQQGPGQQGPYASAAAAAAAGPGQQGPYGPGSSAAAAAAAGSYGYGPGQQGPYGPGASGQNGPGSGQYGPGQQGPGPSAAAAAAAGPGQQGPYGPGASAAAAAAAGSYGPGQQGPGQYGPGSSGPGQQGPYGPGSSAAAAAAAGSYGPGQQGPYGPGPSAAAAAAAGSYQQGPGQQGPYGPGASGPGQQGPYGPGASAAAAAAAGPGQYGPGQQGPSASAAAAAAAGSYGSGPGQYGPYGPGQSGPGSGQQGQGPYGPGASAAAAAAAGSYGPGQQGPYGPGPSAAAAAAAGPGSGQYGPGASGQNGPGSGQYGPGQQGPGPSAAAAAAAGPGSGQQGPGAS

SEQ ID NO: 15 - protein, 2375 aa, Artificial Sequence
  PRT799
MHHHHHHSSGSSGPGQQGPYGPGASAAAAAGQNGPGSGQQGPGQSGQYGPGQQGPGQQGPGSSAAAAAGPGQYGPGQQGPSASAAAAAGPGSGQQGPGASGQYGPGQQGPGQQGPGSSAAAAAGQYGSGPGQQGPYGSAAAAAGPGSGQYGQGPYGPGASGPGQYGPGQQGPSASAAAAAGSGQQGPGQYGPYASAAAAAGQYGSGPGQQGPYGPGQSGSGQQGPGQQGPYASAAAAAGPGQQGPYGPGSSAAAAAGQYGYGPGQQGPYGPGASGQNGPGSGQYGPGQQGPGQSAAAAAGPGQQGPYGPGASAAAAAGQYGPGQQGPGQYGPGSSGPGQQGPYGPGSSAAAAAGQYGPGQQGPYGPGQSAAAAAGQYQQGPGQQGPYGPGASGPGQQGPYGPGASAAAAAGPGQYGPGQQGPSASAAAAAGQYGSGPGQYGPYGPGQSGPGSGQQGQGPYGPGASAAAAAGQYGPGQQGPYGPGQSAAAAAGPGSGQYGPGASGQNGPGSGQYGPGQQGPGQSAAAAAGQYQQGPGQQGPYGPGASAAAAAGQYGSGPGQQGPYGPGQSGSGQQGPGQQGPYASAAAAAGPGSGQQGPGASGQQGPYGPGASAAAAAGQNGPGSGQQGPGQSGQYGPGQQGPGQQGPGSSAAAAAGPGQYGPGQQGPSASAAAAAGPGSGQQGPGASGQYGPGQQGPGQQGPGSSAAAAAGQYGSGPGQQGPYGSAAAAAGPGSGQYGQGPYGPGASGPGQYGPGQQGPSASAAAAAGSGQQGPGQYGPYASAAAAAGQYGSGPGQQGPYGPGQSGSGQQGPGQQGPYASAAAAAGPGQQGPYGPGSSAAAAAGQYGYGPGQQGPYGPGASGQNGPGSGQYGPGQQGPGQSAAAAAGPGQQGPYGPGASAAAAAGQYGPGQQGPGQYGPGSSGPGQQGPYGPGSSAAAAAGQYGPGQQGPYGPGQSAAAAAGQYQQGPGQQGPYGPGASGPGQQGPYGPGASAAAAAGPGQYGPGQQGPSASAAAAAGQYGSGPGQYGPYGPGQSGPGSGQQGQGPYGPGASAAAAAGQYGPGQQGPYGPGQSAAAAAGPGSGQYGPGASGQNGPGSGQYGPGQQGPGQSAAAAAGQYQQGPGQQGPYGPGASAAAAAGQYGSGPGQQGPYGPGQSGSGQQGPGQQGPYASAAAAAGPGSGQQGPGASGQQGPYGPGASAAAAAGQNGPGSGQQGPGQSGQYGPGQQGPGQQGPGSSAAAAAGPGQYGPGQQGPSASAAAAAGPGSGQQGPGASGQYGPGQQGPGQQGPGSSAAAAAGQYGSGPGQQGPYGSAAAAAGPGSGQYGQGPYGPGASGPGQYGPGQQGPSASAAAAAGSGQQGPGQYGPYASAAAAAGQYGSGPGQQGPYGPGQSGSGQQGPGQQGPYASAAAAAGPGQQGPYGPGSSAAAAAGQYGYGPGQQGPYGPGASGQNGPGSGQYGPGQQGPGQSAAAAAGPGQQGPYGPGASAAAAAGQYGPGQQGPGQYGPGSSGPGQQGPYGPGSSAAAAAGQYGPGQQGPYGPGQSAAAAAGQYQQGPGQQGPYGPGASGPGQQGPYGPGASAAAAAGPGQYGPGQQGPSASAAAAAGQYGSGPGQYGPYGPGQSGPGSGQQGQGPYGPGASAAAAAGQYGPGQQGPYGPGQSAAAAAGPGSGQYGPGASGQNGPGSGQYGPGQQGPGQSAAAAAGQYQQGPGQQGPYGPGASAAAAAGQYGSGPGQQGPYGPGQSGSGQQGPGQQGPYASAAAAAGPGSGQQGPGASGQQGPYGPGASAAAAAGQNGPGSGQQGPGQSGQYGPGQQGPGQQGPGSSAAAAAGPGQYGPGQQGPSASAAAAAGPGSGQQGPGASGQYGPGQQGPGQQGPGSSAAAAAGQYGSGPGQQGPYGSAAAAAGPGSGQYGQGPYGPGASGPGQYGPGQQGPSASAAAAAGSGQQGPGQYGPYASAAAAAGQYGSGPGQQGPYGPGQSGSGQQGPGQQGPYASAAAAAGPGQQGPYGPGSSAAAAAGQYGYGPGQQGPYGPGASGQNGPGSGQYGPGQQGPGQSAAAAAGPGQQGPYGPGASAAAAAGQYGPGQQGPGQYGPGSSGPGQQGPYGPGSSAAAAAGQYGPGQQGPYGPGQSAAAAAGQYQQGPGQQGPYGPGASGPGQQGPYGPGASAAAAAGPGQYGPGQQGPSASAAAAAGQYGSGPGQYGPYGPGQSGPGSGQQGQGPYGPGASAAAAAGQYGPGQQGPYGPGQSAAAAAGPGSGQYGPGASGQNGPGSGQYGPGQQGPGQSAAAAAGQYQQGPGQQGPYGPGASAAAAAGQYGSGPGQQGPYGPGQSGSGQQGPGQQGPYASAAAAAGPGSGQQGSSVDKLAAALEHHHHHH

SEQ ID NO: 16 - protein, 608 aa, Artificial Sequence
  PRT313
MHHHHHHSSGSSGPGGQGPYGPGASAAAAAGGNGPGSGQQGPGGSAAAAAGGYGPGGQGPGQQGPGSSAAAAAGPGGYGPGGQGPSASAAAAAGPGSGQQGPGASAAAAAGGYGPGGQGPGQQGPGSSAAAAAGGYGSGPGQQGPYGSAAAAAGPGSGGYGQGPYGPGASAAAAAGPGGYGPGGQGPSASAAAAAGSGQQGPGGYGPYASAAAAAGGYGSGPGQQGPYGPGGSAAAAAGSGQQGPGQQGPYASAAAAAGPGGQGPYGPGSSAAAAAGGYGYGPGGQGPYGPGASAAAAAGGNGPGSGGYGPGQQGPGGSAAAAAGPGGQGPYGPGASAAAAAGGYGPGGQGPGGYGPGSSAAAAAGPGGQGPYGPGSSAAAAAGGYGPGQQGPYGPGGSAAAAAGGYQQGPGGQGPYGPGASAAAAAGPGGQGPYGPGASAAAAAGPGGYGPGGQGPSASAAAAAGGYGSGPGGYGPYGPGGSAAAAAGPGSGQQGQGPYGPGASAAAAAGGYGPGQQGPYGPGGSAAAAAGPGSGGYGPGASAAAAAGGNGPGSGGYGPGQQGPGGSAAAAAGGYQQGPGGQGPYGPGASAAAAAGPGSGQQGPGAS

SEQ ID NO: 17 - protein, 590 aa, Artificial Sequence
  Met-PRT399
MGPGGQGPYGPGASAAAAAGGNGPGSGQQGPGGSGGYGPGGQGPGQQGPGSSAAAAAGPGGYGPGGQGPSASAAAAAGPGSGQQGPGASGGYGPGGQGPGQQGPGSSAAAAAGGYGSGPGQQGPYGSAAAAAGPGSGGYGQGPYGPGASGPGGYGPGGQGPSASAAAAAGSGQQGPGGYGPYASAAAAAGGYGSGPGQQGPYGPGGSGSGQQGPGQQGPYASAAAAAGPGGQGPYGPGSSAAAAAGGYGYGPGGQGPYGPGASGGNGPGSGGYGPGQQGPGGSAAAAAGPGGQGPYGPGASAAAAAGGYGPGGQGPGGYGPGSSGPGGQGPYGPGSSAAAAAGGYGPGQQGPYGPGGSAAAAAGGYQQGPGGQGPYGPGASGPGGQGPYGPGASAAAAAGPGGYGPGGQGPSASAAAAAGGYGSGPGGYGPYGPGGSGPGSGQQGQGPYGPGASAAAAAGGYGPGQQGPYGPGGSAAAAAGPGSGGYGPGASGGNGPGSGGYGPGQQGPGGSAAAAAGGYQQGPGGQGPYGPGASAAAAAGGYGSGPGQQGPYGPGGSGSGQQGPGQQGPYASAAAAAGPGSGQQGPGAS

SEQ ID NO: 18 - protein, 601 aa, Artificial Sequence
  PRT399
MHHHHHHSSGSSGPGGQGPYGPGASAAAAAGGNGPGSGQQGPGGSGGYGPGGQGPGQQGPGSSAAAAAGPGGYGPGGQGPSASAAAAAGPGSGQQGPGASGGYGPGGQGPGQQGPGSSAAAAAGGYGSGPGQQGPYGSAAAAAGPGSGGYGQGPYGPGASGPGGYGPGGQGPSASAAAAAGSGQQGPGGYGPYASAAAAAGGYGSGPGQQGPYGPGGSGSGQQGPGQQGPYASAAAAAGPGGQGPYGPGSSAAAAAGGYGYGPGGQGPYGPGASGGNGPGSGGYGPGQQGPGGSAAAAAGPGGQGPYGPGASAAAAAGGYGPGGQGPGGYGPGSSGPGGQGPYGPGSSAAAAAGGYGPGQQGPYGPGGSAAAAAGGYQQGPGGQGPYGPGASGPGGQGPYGPGASAAAAAGPGGYGPGGQGPSASAAAAAGGYGSGPGGYGPYGPGGSGPGSGQQGQGPYGPGASAAAAAGGYGPGQQGPYGPGGSAAAAAGPGSGGYGPGASGGNGPGSGGYGPGQQGPGGSAAAAAGGYQQGPGGQGPYGPGASAAAAAGGYGSGPGQQGPYGPGGSGSGQQGPGQQGPYASAAAAAGPGSGQQGPGAS

SEQ ID NO: 19 - protein, 612 aa, Artificial Sequence
  Met-PRT720
MGPGQQGPYGPGASAAAAAGQNGPGSGQQGPGQSGQYGPGQQGPGQQGPGSSAAAAAGPGQYVLIGPGQQVLIGPSASAAAAAGPGSGQQGPGASGQYGPGQQGPGQQGPGSSAAAAAGSYGSVLIGPGQQVLIGPYGSAAAAAGPGSGQYGQGPYGPGASGPGQYGPGQQGPSASAAAAAGSGQQVLIGPGQYVLIGPYASAAAAAGQYGSGPGQQGPYGPGQSGSGQQGPGQQGPYASAAAAAGPGQQVLIGPYVLIGPGSSAAAAAGQYGYGPGQQGPYGPGASGQNGPGSGQYGPGQQGPGQSAAAAAGPGQQVLIGPYVLIGPGASAAAAAGQYGPGQQGPGQYGPGSSGPGQQGPYGPGSSAAAAAGSYGPGQQVLIGPYVLIGPGPSAAAAAGQYQQGPGQQGPYGPGASGPGQQGPYGPGASAAAAAGPGQYVLIGPGQQVLIGPSASAAAAAGQYGSGPGQYGPYGPGQSGPGSGQQGQGPYGPGASAAAAAGSYGPGQQVLIGPYVLIGPGPSAAAAAGPGSGQYGPGASGQNGPGSGQYGPGQQGPGQSAAAAAGQYQQVLIGPGQQGPYVLIGPGASAAAAAGPGSGQQVLIGPGASVLI

SEQ ID NO: 20 - protein, 592 aa, Artificial Sequence
  Met-PRT665
MGPGQQGPYGPGASAAAAAAAGSNGPGSGQQGPGQSGQYGPGQQGPGQQGPGSSAAAAAAAGPGQYVLIGPGQQGPSASAAAAAAAGPGSGQQGPGASGQYGPGQQGPGQQGPGSSAAAAAAAGSYGSVLIGPGQQGPYGSAAAAAAAGPGSGQYGQGPYGPGASGPGQYGPGQQGPSASAAAAAAAGSGQQVLIGPGQYGPYASAAAAAAAGSYGSGPGQQGPYGPGQSGSGQQGPGQQGPYASAAAAAAAGPGQQVLIGPYGPGSSAAAAAAAGSYGYGPGQQGPYGPGASGQNGPGSGQYGPGQQGPGPSAAAAAAAGPGQQVLIGPYGPGASAAAAAAAGSYGPGQQGPGQYGPGSSGPGQQGPYGPGSSAAAAAAAGSYGPGQQVLIGPYGPGPSAAAAAAAGSYQQGPGQQGPYGPGASGPGQQGPYGPGASAAAAAAAGPGQYVLIGPGQQGPSASAAAAAAAGSYGSGPGQYGPYGPGQSGPGSGQQGQGPYGPGASAAAAAAAGSYGPGQQVLIGPYGPGPSAAAAAAAGPGSGQYGPGASGQNGPGSGQYGPGQQGPGPSAAAAAAAGPGSGQQGPGASVLI

SEQ ID NO: 21 - protein, 619 aa, Artificial Sequence
  Met-PRT666
MGPGQQGPYGPGASAAAAAAAGSNGPGSGQQGPGQSGQYGPGQQGPGQQGPGSSAAAAAAAGPGQYVLIGPGQQVLIGPSASAAAAAAAGPGSGQQGPGASGQYGPGQQGPGQQGPGSSAAAAAAAGSYGSVLIGPGQQVLIGPYGSAAAAAAAGPGSGQYGQGPYGPGASGPGQYGPGQQGPSASAAAAAAAGSGQQVLIGPGQYVLIGPYASAAAAAAAGSYGSGPGQQGPYGPGQSGSGQQGPGQQGPYASAAAAAAAGPGQQVLIGPYVLIGPGSSAAAAAAAGSYGYGPGQQGPYGPGASGQNGPGSGQYGPGQQGPGPSAAAAAAAGPGQQVLIGPYVLIGPGASAAAAAAAGSYGPGQQGPGQYGPGSSGPGQQGPYGPGSSAAAAAAAGSYGPGQQVLIGPYVLIGPGPSAAAAAAAGSYQQGPGQQGPYGPGASGPGQQGPYGPGASAAAAAAAGPGQYVLIGPGQQVLIGPSASAAAAAAAGSYGSGPGQYGPYGPGQSGPGSGQQGQGPYGPGASAAAAAAAGSYGPGQQVLIGPYVLIGPGPSAAAAAAAGPGSGQYGPGASGQNGPGSGQYGPGQQGPGPSAAAAAAAGPGSGQQVLIGPGASVLI

SEQ ID NO: 22 - protein, 623 aa, Artificial Sequence
  PRT720
MHHHHHHSSGSSGPGQQGPYGPGASAAAAAGQNGPGSGQQGPGQSGQYGPGQQGPGQQGPGSSAAAAAGPGQYVLIGPGQQVLIGPSASAAAAAGPGSGQQGPGASGQYGPGQQGPGQQGPGSSAAAAAGSYGSVLIGPGQQVLIGPYGSAAAAAGPGSGQYGQGPYGPGASGPGQYGPGQQGPSASAAAAAGSGQQVLIGPGQYVLIGPYASAAAAAGQYGSGPGQQGPYGPGQSGSGQQGPGQQGPYASAAAAAGPGQQVLIGPYVLIGPGSSAAAAAGQYGYGPGQQGPYGPGASGQNGPGSGQYGPGQQGPGQSAAAAAGPGQQVLIGPYVLIGPGASAAAAAGQYGPGQQGPGQYGPGSSGPGQQGPYGPGSSAAAAAGSYGPGQQVLIGPYVLIGPGPSAAAAAGQYQQGPGQQGPYGPGASGPGQQGPYGPGASAAAAAGPGQYVLIGPGQQVLIGPSASAAAAAGQYGSGPGQYGPYGPGQSGPGSGQQGQGPYGPGASAAAAAGSYGPGQQVLIGPYVLIGPGPSAAAAAGPGSGQYGPGASGQNGPGSGQYGPGQQGPGQSAAAAAGQYQQVLIGPGQQGPYVLIGPGASAAAAAGPGSGQQVLIGPGASVLI

SEQ ID NO: 23 - protein, 603 aa, Artificial Sequence
  PRT665
MHHHHHHSSGSSGPGQQGPYGPGASAAAAAAAGSNGPGSGQQGPGQSGQYGPGQQGPGQQGPGSSAAAAAAAGPGQYVLIGPGQQGPSASAAAAAAAGPGSGQQGPGASGQYGPGQQGPGQQGPGSSAAAAAAAGSYGSVLIGPGQQGPYGSAAAAAAAGPGSGQYGQGPYGPGASGPGQYGPGQQGPSASAAAAAAAGSGQQVLIGPGQYGPYASAAAAAAAGSYGSGPGQQGPYGPGQSGSGQQGPGQQGPYASAAAAAAAGPGQQVLIGPYGPGSSAAAAAAAGSYGYGPGQQGPYGPGASGQNGPGSGQYGPGQQGPGPSAAAAAAAGPGQQVLIGPYGPGASAAAAAAAGSYGPGQQGPGQYGPGSSGPGQQGPYGPGSSAAAAAAAGSYGPGQQVLIGPYGPGPSAAAAAAAGSYQQGPGQQGPYGPGASGPGQQGPYGPGASAAAAAAAGPGQYVLIGPGQQGPSASAAAAAAAGSYGSGPGQYGPYGPGQSGPGSGQQGQGPYGPGASAAAAAAAGSYGPGQQVLIGPYGPGPSAAAAAAAGPGSGQYGPGASGQNGPGSGQYGPGQQGPGPSAAAAAAAGPGSGQQGPGASVLI

SEQ ID NO: 24 - protein, 630 aa, Artificial Sequence
  PRT666
MHHHHHHSSGSSGPGQQGPYGPGASAAAAAAAGSNGPGSGQQGPGQSGQYGPGQQGPGQQGPGSSAAAAAAAGPGQYVLIGPGQQVLIGPSASAAAAAAAGPGSGQQGPGASGQYGPGQQGPGQQGPGSSAAAAAAAGSYGSVLIGPGQQVLIGPYGSAAAAAAAGPGSGQYGQGPYGPGASGPGQYGPGQQGPSASAAAAAAAGSGQQVLIGPGQYVLIGPYASAAAAAAAGSYGSGPGQQGPYGPGQSGSGQQGPGQQGPYASAAAAAAAGPGQQVLIGPYVLIGPGSSAAAAAAAGSYGYGPGQQGPYGPGASGQNGPGSGQYGPGQQGPGPSAAAAAAAGPGQQVLIGPYVLIGPGASAAAAAAAGSYGPGQQGPGQYGPGSSGPGQQGPYGPGSSAAAAAAAGSYGPGQQVLIGPYVLIGPGPSAAAAAAAGSYQQGPGQQGPYGPGASGPGQQGPYGPGASAAAAAAAGPGQYVLIGPGQQVLIGPSASAAAAAAAGSYGSGPGQYGPYGPGQSGPGSGQQGQGPYGPGASAAAAAAAGSYGPGQQVLIGPYVLIGPGPSAAAAAAAGPGSGQYGPGASGQNGPGSGQYGPGQQGPGPSAAAAAAAGPGSGQQVLIGPGASVLI

SEQ ID NO: 25 - protein, 593 aa, Artificial Sequence
  M_PRT888
MGSSGPGVLGPYGPGASAAAAAGQNGPGSGVLGPGQSGQYGPGVLGPGVLGPGSSAAAAAGPGQYGPGVLGPSASAAAAAGPGSGVLGPGASGQYGPGVLGPGVLGPGSSAAAAAGQYGSGPGVLGPYGSAAAAAGPGSGQYGQGPYGPGASGPGQYGPGVLGPSASAAAAAGSGVLGPGQYGPYASAAAAAGQYGSGPGVLGPYGPGQSGSGVLGPGVLGPYASAAAAAGPGVLGPYGPGSSAAAAAGQYGYGPGVLGPYGPGASGQNGPGSGQYGPGVLGPGQSAAAAAGPGVLGPYGPGASAAAAAGQYGPGVLGPGQYGPGSSGPGVLGPYGPGSSAAAAAGQYGPGVLGPYGPGQSAAAAAGQYVLGPGVLGPYGPGASGPGVLGPYGPGASAAAAAGPGQYGPGVLGPSASAAAAAGQYGSGPGQYGPYGPGQSGPGSGVLGQGPYGPGASAAAAAGQYGPGVLGPYGPGQSAAAAAGPGSGQYGPGASGQNGPGSGQYGPGVLGPGQSAAAAAGQYVLGPGVLGPYGPGASAAAAAGQYGSGPGVLGPYGPGQSGSGVLGPGVLGPYASAAAAAGPGSGVLGPGAS

SEQ ID NO: 26 - protein, 590 aa, Artificial Sequence
  M_PRT965
MGPGTSGPYGPGASAAAAAGANGPGSGTSGPGASGAYGPGTSGPGTSGPGSSAAAAAGPGAYGPGTSGPSASAAAAAGPGSGTSGPGASGAYGPGTSGPGTSGPGSSAAAAAGAYGSGPGTSGPYGSAAAAAGPGSGAYGAGPYGPGASGPGAYGPGTSGPSASAAAAAGSGTSGPGAYGPYASAAAAAGAYGSGPGTSGPYGPGASGSGTSGPGTSGPYASAAAAAGPGTSGPYGPGSSAAAAAGAYGYGPGTSGPYGPGASGANGPGSGAYGPGTSGPGASAAAAAGPGTSGPYGPGASAAAAAGAYGPGTSGPGAYGPGSSGPGTSGPYGPGSSAAAAAGAYGPGTSGPYGPGASAAAAAGAYTSGPGTSGPYGPGASGPGTSGPYGPGASAAAAAGPGAYGPGTSGPSASAAAAAGAYGSGPGAYGPYGPGASGPGSGTSGAGPYGPGASAAAAAGAYGPGTSGPYGPGASAAAAAGPGSGAYGPGASGANGPGSGAYGPGTSGPGASAAAAAGAYTSGPGTSGPYGPGASAAAAAGAYGSGPGTSGPYGPGASGSGTSGPGTSGPYASAAAAAGPGSGTSGPGAS

SEQ ID NO: 27 - protein, 593 aa, Artificial Sequence
  M_PRT889
MGSSGPGVLGPYGPGASAAAAAGINGPGSGVLGPGISGIYGPGVLGPGVLGPGSSAAAAAGPGIYGPGVLGPSASAAAAAGPGSGVLGPGASGIYGPGVLGPGVLGPGSSAAAAAGIYGSGPGVLGPYGSAAAAAGPGSGIYGIGPYGPGASGPGIYGPGVLGPSASAAAAAGSGVLGPGIYGPYASAAAAAGIYGSGPGVLGPYGPGISGSGVLGPGVLGPYASAAAAAGPGVLGPYGPGSSAAAAAGIYGYGPGVLGPYGPGASGINGPGSGIYGPGVLGPGISAAAAAGPGVLGPYGPGASAAAAAGIYGPGVLGPGIYGPGSSGPGVLGPYGPGSSAAAAAGIYGPGVLGPYGPGISAAAAAGIYVLGPGVLGPYGPGASGPGVLGPYGPGASAAAAAGPGIYGPGVLGPSASAAAAAGIYGSGPGIYGPYGPGISGPGSGVLGIGPYGPGASAAAAAGIYGPGVLGPYGPGISAAAAAGPGSGIYGPGASGINGPGSGIYGPGVLGPGISAAAAAGIYVLGPGVLGPYGPGASAAAAAGIYGSGPGVLGPYGPGISGSGVLGPGVLGPYASAAAAAGPGSGVLGPGAS

SEQ ID NO: 28 - protein, 590 aa, Artificial Sequence
  M_PRT916
MGPGVIGPYGPGASAAAAAGLNGPGSGVIGPGLSGLYGPGVIGPGVIGPGSSAAAAAGPGLYGPGVIGPSASAAAAAGPGSGVIGPGASGLYGPGVIGPGVIGPGSSAAAAAGLYGSGPGVIGPYGSAAAAAGPGSGLYGLGPYGPGASGPGLYGPGVIGPSASAAAAAGSGVIGPGLYGPYASAAAAAGLYGSGPGVIGPYGPGLSGSGVIGPGVIGPYASAAAAAGPGVIGPYGPGSSAAAAAGLYGYGPGVIGPYGPGASGLNGPGSGLYGPGVIGPGLSAAAAAGPGVIGPYGPGASAAAAAGLYGPGVIGPGLYGPGSSGPGVIGPYGPGSSAAAAAGLYGPGVIGPYGPGLSAAAAAGLYVIGPGVIGPYGPGASGPGVIGPYGPGASAAAAAGPGLYGPGVIGPSASAAAAAGLYGSGPGLYGPYGPGLSGPGSGVIGLGPYGPGASAAAAAGLYGPGVIGPYGPGLSAAAAAGPGSGLYGPGASGLNGPGSGLYGPGVIGPGLSAAAAAGLYVIGPGVIGPYGPGASAAAAAGLYGSGPGVIGPYGPGLSGSGVIGPGVIGPYASAAAAAGPGSGVIGPGAS

SEQ ID NO: 29 - protein, 590 aa, Artificial Sequence
  M_ PRT918
MGPGVFGPYGPGASAAAAAGINGPGSGVFGPGISGIYGPGVFGPGVFGPGSSAAAAAGPGIYGPGVFGPSASAAAAAGPGSGVFGPGASGIYGPGVFGPGVFGPGSSAAAAAGIYGSGPGVFGPYGSAAAAAGPGSGIYGIGPYGPGASGPGIYGPGVFGPSASAAAAAGSGVFGPGIYGPYASAAAAAGIYGSGPGVFGPYGPGISGSGVFGPGVFGPYASAAAAAGPGVFGPYGPGSSAAAAAGIYGYGPGVFGPYGPGASGINGPGSGIYGPGVFGPGISAAAAAGPGVFGPYGPGASAAAAAGIYGPGVFGPGIYGPGSSGPGVFGPYGPGSSAAAAAGIYGPGVFGPYGPGISAAAAAGIYVFGPGVFGPYGPGASGPGVFGPYGPGASAAAAAGPGIYGPGVFGPSASAAAAAGIYGSGPGIYGPYGPGISGPGSGVFGIGPYGPGASAAAAAGIYGPGVFGPYGPGISAAAAAGPGSGIYGPGASGINGPGSGIYGPGVFGPGISAAAAAGIYVFGPGVFGPYGPGASAAAAAGIYGSGPGVFGPYGPGISGSGVFGPGVFGPYASAAAAAGPGSGVFGPGAS

SEQ ID NO: 30 - protein, 565 aa, Artificial Sequence
  M_PRT699
MGPGVLGPYGPGASAAAAAAAGSNGPGSGVLGPGQSGQYGPGVLGPGVLGPGSSAAAAAAAGPGQYGPGVLGPSASAAAAAAAGPGSGVLGPGASGQYGPGVLGPGVLGPGSSAAAAAAAGSYGSGPGVLGPYGSAAAAAAAGPGSGQYGQGPYGPGASGPGQYGPGVLGPSASAAAAAAAGSGVLGPGQYGPYASAAAAAAAGSYGSGPGVLGPYGPGQSGSGVLGPGVLGPYASAAAAAAAGPGVLGPYGPGSSAAAAAAAGSYGYGPGVLGPYGPGASGQNGPGSGQYGPGVLGPGPSAAAAAAAGPGVLGPYGPGASAAAAAAAGSYGPGVLGPGQYGPGSSGPGVLGPYGPGSSAAAAAAAGSYGPGVLGPYGPGPSAAAAAAAGSYVLGPGVLGPYGPGASGPGVLGPYGPGASAAAAAAAGPGQYGPGVLGPSASAAAAAAAGSYGSGPGQYGPYGPGQSGPGSGVLGQGPYGPGASAAAAAAAGSYGPGVLGPYGPGPSAAAAAAAGPGSGQYGPGASGQNGPGSGQYGPGVLGPGPSAAAAAAAGPGSGVLGPGAS

SEQ ID NO: 31 - protein, 565 aa, Artificial Sequence
  M_PRT698
MGPGVLGPYGPGASAAAAAAAGSNGPGSGVLGPGISGIYGPGVLGPGVLGPGSSAAAAAAAGPGIYGPGVLGPSASAAAAAAAGPGSGVLGPGASGIYGPGVLGPGVLGPGSSAAAAAAAGSYGSGPGVLGPYGSAAAAAAAGPGSGIYGIGPYGPGASGPGIYGPGVLGPSASAAAAAAAGSGVLGPGIYGPYASAAAAAAAGSYGSGPGVLGPYGPGISGSGVLGPGVLGPYASAAAAAAAGPGVLGPYGPGSSAAAAAAAGSYGYGPGVLGPYGPGASGINGPGSGIYGPGVLGPGPSAAAAAAAGPGVLGPYGPGASAAAAAAAGSYGPGVLGPGIYGPGSSGPGVLGPYGPGSSAAAAAAAGSYGPGVLGPYGPGPSAAAAAAAGSYVLGPGVLGPYGPGASGPGVLGPYGPGASAAAAAAAGPGIYGPGVLGPSASAAAAAAAGSYGSGPGIYGPYGPGISGPGSGVLGIGPYGPGASAAAAAAAGSYGPGVLGPYGPGPSAAAAAAAGPGSGIYGPGASGINGPGSGIYGPGVLGPGPSAAAAAAAGPGSGVLGPGAS

SEQ ID NO: 32 - protein, 1179 aa, Artificial Sequence
  Met-PRT966
MGPGVFGPYGPGASAAAAAGINGPGSGVFGPGISGIYGPGVFGPGVFGPGSSAAAAAGPGIYGPGVFGPSASAAAAAGPGSGVFGPGASGIYGPGVFGPGVFGPGSSAAAAAGIYGSGPGVFGPYGSAAAAAGPGSGIYGIGPYGPGASGPGIYGPGVFGPSASAAAAAGSGVFGPGIYGPYASAAAAAGIYGSGPGVFGPYGPGISGSGVFGPGVFGPYASAAAAAGPGVFGPYGPGSSAAAAAGIYGYGPGVFGPYGPGASGINGPGSGIYGPGVFGPGISAAAAAGPGVFGPYGPGASAAAAAGIYGPGVFGPGIYGPGSSGPGVFGPYGPGSSAAAAAGIYGPGVFGPYGPGISAAAAAGIYVFGPGVFGPYGPGASGPGVFGPYGPGASAAAAAGPGIYGPGVFGPSASAAAAAGIYGSGPGIYGPYGPGISGPGSGVFGIGPYGPGASAAAAAGIYGPGVFGPYGPGISAAAAAGPGSGIYGPGASGINGPGSGIYGPGVFGPGISAAAAAGIYVFGPGVFGPYGPGASAAAAAGIYGSGPGVFGPYGPGISGSGVFGPGVFGPYASAAAAAGPGSGVFGPGASGPGVFGPYGPGASAAAAAGINGPGSGVFGPGISGIYGPGVFGPGVFGPGSSAAAAAGPGIYGPGVFGPSASAAAAAGPGSGVFGPGASGIYGPGVFGPGVFGPGSSAAAAAGIYGSGPGVFGPYGSAAAAAGPGSGIYGIGPYGPGASGPGIYGPGVFGPSASAAAAAGSGVFGPGIYGPYASAAAAAGIYGSGPGVFGPYGPGISGSGVFGPGVFGPYASAAAAAGPGVFGPYGPGSSAAAAAGIYGYGPGVFGPYGPGASGINGPGSGIYGPGVFGPGISAAAAAGPGVFGPYGPGASAAAAAGIYGPGVFGPGIYGPGSSGPGVFGPYGPGSSAAAAAGIYGPGVFGPYGPGISAAAAAGIYVFGPGVFGPYGPGASGPGVFGPYGPGASAAAAAGPGIYGPGVFGPSASAAAAAGIYGSGPGIYGPYGPGISGPGSGVFGIGPYGPGASAAAAAGIYGPGVFGPYGPGISAAAAAGPGSGIYGPGASGINGPGSGIYGPGVFGPGISAAAAAGIYVFGPGVFGPYGPGASAAAAAGIYGSGPGVFGPYGPGISGSGVFGPGVFGPYASAAAAAGPGSGVFGPGAS

SEQ ID NO: 33 - protein, 601 aa, Artificial Sequence
  PRT888
MHHHHHHSSGSSGPGVLGPYGPGASAAAAAGQNGPGSGVLGPGQSGQYGPGVLGPGVLGPGSSAAAAAGPGQYGPGVLGPSASAAAAAGPGSGVLGPGASGQYGPGVLGPGVLGPGSSAAAAAGQYGSGPGVLGPYGSAAAAAGPGSGQYGQGPYGPGASGPGQYGPGVLGPSASAAAAAGSGVLGPGQYGPYASAAAAAGQYGSGPGVLGPYGPGQSGSGVLGPGVLGPYASAAAAAGPGVLGPYGPGSSAAAAAGQYGYGPGVLGPYGPGASGQNGPGSGQYGPGVLGPGQSAAAAAGPGVLGPYGPGASAAAAAGQYGPGVLGPGQYGPGSSGPGVLGPYGPGSSAAAAAGQYGPGVLGPYGPGQSAAAAAGQYVLGPGVLGPYGPGASGPGVLGPYGPGASAAAAAGPGQYGPGVLGPSASAAAAAGQYGSGPGQYGPYGPGQSGPGSGVLGQGPYGPGASAAAAAGQYGPGVLGPYGPGQSAAAAAGPGSGQYGPGASGQNGPGSGQYGPGVLGPGQSAAAAAGQYVLGPGVLGPYGPGASAAAAAGQYGSGPGVLGPYGPGQSGSGVLGPGVLGPYASAAAAAGPGSGVLGPGAS

SEQ ID NO: 34 - protein, 601 aa, Artificial Sequence
  PRT965
MHHHHHHSSGSSGPGTSGPYGPGASAAAAAGANGPGSGTSGPGASGAYGPGTSGPGTSGPGSSAAAAAGPGAYGPGTSGPSASAAAAAGPGSGTSGPGASGAYGPGTSGPGTSGPGSSAAAAAGAYGSGPGTSGPYGSAAAAAGPGSGAYGAGPYGPGASGPGAYGPGTSGPSASAAAAAGSGTSGPGAYGPYASAAAAAGAYGSGPGTSGPYGPGASGSGTSGPGTSGPYASAAAAAGPGTSGPYGPGSSAAAAAGAYGYGPGTSGPYGPGASGANGPGSGAYGPGTSGPGASAAAAAGPGTSGPYGPGASAAAAAGAYGPGTSGPGAYGPGSSGPGTSGPYGPGSSAAAAAGAYGPGTSGPYGPGASAAAAAGAYTSGPGTSGPYGPGASGPGTSGPYGPGASAAAAAGPGAYGPGTSGPSASAAAAAGAYGSGPGAYGPYGPGASGPGSGTSGAGPYGPGASAAAAAGAYGPGTSGPYGPGASAAAAAGPGSGAYGPGASGANGPGSGAYGPGTSGPGASAAAAAGAYTSGPGTSGPYGPGASAAAAAGAYGSGPGTSGPYGPGASGSGTSGPGTSGPYASAAAAAGPGSGTSGPGAS

SEQ ID NO: 35 - protein, 601 aa, Artificial Sequence
  PRT889
MHHHHHHSSGSSGPGVLGPYGPGASAAAAAGINGPGSGVLGPGISGIYGPGVLGPGVLGPGSSAAAAAGPGIYGPGVLGPSASAAAAAGPGSGVLGPGASGIYGPGVLGPGVLGPGSSAAAAAGIYGSGPGVLGPYGSAAAAAGPGSGIYGIGPYGPGASGPGIYGPGVLGPSASAAAAAGSGVLGPGIYGPYASAAAAAGIYGSGPGVLGPYGPGISGSGVLGPGVLGPYASAAAAAGPGVLGPYGPGSSAAAAAGIYGYGPGVLGPYGPGASGINGPGSGIYGPGVLGPGISAAAAAGPGVLGPYGPGASAAAAAGIYGPGVLGPGIYGPGSSGPGVLGPYGPGSSAAAAAGIYGPGVLGPYGPGISAAAAAGIYVLGPGVLGPYGPGASGPGVLGPYGPGASAAAAAGPGIYGPGVLGPSASAAAAAGIYGSGPGIYGPYGPGISGPGSGVLGIGPYGPGASAAAAAGIYGPGVLGPYGPGISAAAAAGPGSGIYGPGASGINGPGSGIYGPGVLGPGISAAAAAGIYVLGPGVLGPYGPGASAAAAAGIYGSGPGVLGPYGPGISGSGVLGPGVLGPYASAAAAAGPGSGVLGPGAS

SEQ ID NO: 36 - protein, 601 aa, Artificial Sequence
  PRT916
MHHHHHHSSGSSGPGVIGPYGPGASAAAAAGLNGPGSGVIGPGLSGLYGPGVIGPGVIGPGSSAAAAAGPGLYGPGVIGPSASAAAAAGPGSGVIGPGASGLYGPGVIGPGVIGPGSSAAAAAGLYGSGPGVIGPYGSAAAAAGPGSGLYGLGPYGPGASGPGLYGPGVIGPSASAAAAAGSGVIGPGLYGPYASAAAAAGLYGSGPGVIGPYGPGLSGSGVIGPGVIGPYASAAAAAGPGVIGPYGPGSSAAAAAGLYGYGPGVIGPYGPGASGLNGPGSGLYGPGVIGPGLSAAAAAGPGVIGPYGPGASAAAAAGLYGPGVIGPGLYGPGSSGPGVIGPYGPGSSAAAAAGLYGPGVIGPYGPGLSAAAAAGLYVIGPGVIGPYGPGASGPGVIGPYGPGASAAAAAGPGLYGPGVIGPSASAAAAAGLYGSGPGLYGPYGPGLSGPGSGVIGLGPYGPGASAAAAAGLYGPGVIGPYGPGLSAAAAAGPGSGLYGPGASGLNGPGSGLYGPGVIGPGLSAAAAAGLYVIGPGVIGPYGPGASAAAAAGLYGSGPGVIGPYGPGLSGSGVIGPGVIGPYASAAAAAGPGSGVIGPGAS

SEQ ID NO: 37 - protein, 601 aa, Artificial Sequence
  PRT918
MHHHHHHSSGSSGPGVFGPYGPGASAAAAAGINGPGSGVFGPGISGIYGPGVFGPGVFGPGSSAAAAAGPGIYGPGVFGPSASAAAAAGPGSGVFGPGASGIYGPGVFGPGVFGPGSSAAAAAGIYGSGPGVFGPYGSAAAAAGPGSGIYGIGPYGPGASGPGIYGPGVFGPSASAAAAAGSGVFGPGIYGPYASAAAAAGIYGSGPGVFGPYGPGISGSGVFGPGVFGPYASAAAAAGPGVFGPYGPGSSAAAAAGIYGYGPGVFGPYGPGASGINGPGSGIYGPGVFGPGISAAAAAGPGVFGPYGPGASAAAAAGIYGPGVFGPGIYGPGSSGPGVFGPYGPGSSAAAAAGIYGPGVFGPYGPGISAAAAAGIYVFGPGVFGPYGPGASGPGVFGPYGPGASAAAAAGPGIYGPGVFGPSASAAAAAGIYGSGPGIYGPYGPGISGPGSGVFGIGPYGPGASAAAAAGIYGPGVFGPYGPGISAAAAAGPGSGIYGPGASGINGPGSGIYGPGVFGPGISAAAAAGIYVFGPGVFGPYGPGASAAAAAGIYGSGPGVFGPYGPGISGSGVFGPGVFGPYASAAAAAGPGSGVFGPGAS

SEQ ID NO: 38 - protein, 576 aa, Artificial Sequence
  PRT699
MHHHHHHSSGSSGPGVLGPYGPGASAAAAAAAGSNGPGSGVLGPGQSGQYGPGVLGPGVLGPGSSAAAAAAAGPGQYGPGVLGPSASAAAAAAAGPGSGVLGPGASGQYGPGVLGPGVLGPGSSAAAAAAAGSYGSGPGVLGPYGSAAAAAAAGPGSGQYGQGPYGPGASGPGQYGPGVLGPSASAAAAAAAGSGVLGPGQYGPYASAAAAAAAGSYGSGPGVLGPYGPGQSGSGVLGPGVLGPYASAAAAAAAGPGVLGPYGPGSSAAAAAAAGSYGYGPGVLGPYGPGASGQNGPGSGQYGPGVLGPGPSAAAAAAAGPGVLGPYGPGASAAAAAAAGSYGPGVLGPGQYGPGSSGPGVLGPYGPGSSAAAAAAAGSYGPGVLGPYGPGPSAAAAAAAGSYVLGPGVLGPYGPGASGPGVLGPYGPGASAAAAAAAGPGQYGPGVLGPSASAAAAAAAGSYGSGPGQYGPYGPGQSGPGSGVLGQGPYGPGASAAAAAAAGSYGPGVLGPYGPGPSAAAAAAAGPGSGQYGPGASGQNGPGSGQYGPGVLGPGPSAAAAAAAGPGSGVLGPGAS

SEQ ID NO: 39 - protein, 576 aa, Artificial Sequence
  PRT698
MHHHHHHSSGSSGPGVLGPYGPGASAAAAAAAGSNGPGSGVLGPGISGIYGPGVLGPGVLGPGSSAAAAAAAGPGIYGPGVLGPSASAAAAAAAGPGSGVLGPGASGIYGPGVLGPGVLGPGSSAAAAAAAGSYGSGPGVLGPYGSAAAAAAAGPGSGIYGIGPYGPGASGPGIYGPGVLGPSASAAAAAAAGSGVLGPGIYGPYASAAAAAAAGSYGSGPGVLGPYGPGISGSGVLGPGVLGPYASAAAAAAAGPGVLGPYGPGSSAAAAAAAGSYGYGPGVLGPYGPGASGINGPGSGIYGPGVLGPGPSAAAAAAAGPGVLGPYGPGASAAAAAAAGSYGPGVLGPGIYGPGSSGPGVLGPYGPGSSAAAAAAAGSYGPGVLGPYGPGPSAAAAAAAGSYVLGPGVLGPYGPGASGPGVLGPYGPGASAAAAAAAGPGIYGPGVLGPSASAAAAAAAGSYGSGPGIYGPYGPGISGPGSGVLGIGPYGPGASAAAAAAAGSYGPGVLGPYGPGPSAAAAAAAGPGSGIYGPGASGINGPGSGIYGPGVLGPGPSAAAAAAAGPGSGVLGPGAS

SEQ ID NO: 40 - protein, 1190 aa, Artificial Sequence
  PRT966
MHHHHHHSSGSSGPGVFGPYGPGASAAAAAGINGPGSGVFGPGISGIYGPGVFGPGVFGPGSSAAAAAGPGIYGPGVFGPSASAAAAAGPGSGVFGPGASGIYGPGVFGPGVFGPGSSAAAAAGIYGSGPGVFGPYGSAAAAAGPGSGIYGIGPYGPGASGPGIYGPGVFGPSASAAAAAGSGVFGPGIYGPYASAAAAAGIYGSGPGVFGPYGPGISGSGVFGPGVFGPYASAAAAAGPGVFGPYGPGSSAAAAAGIYGYGPGVFGPYGPGASGINGPGSGIYGPGVFGPGISAAAAAGPGVFGPYGPGASAAAAAGIYGPGVFGPGIYGPGSSGPGVFGPYGPGSSAAAAAGIYGPGVFGPYGPGISAAAAAGIYVFGPGVFGPYGPGASGPGVFGPYGPGASAAAAAGPGIYGPGVFGPSASAAAAAGIYGSGPGIYGPYGPGISGPGSGVFGIGPYGPGASAAAAAGIYGPGVFGPYGPGISAAAAAGPGSGIYGPGASGINGPGSGIYGPGVFGPGISAAAAAGIYVFGPGVFGPYGPGASAAAAAGIYGSGPGVFGPYGPGISGSGVFGPGVFGPYASAAAAAGPGSGVFGPGASGPGVFGPYGPGASAAAAAGINGPGSGVFGPGISGIYGPGVFGPGVFGPGSSAAAAAGPGIYGPGVFGPSASAAAAAGPGSGVFGPGASGIYGPGVFGPGVFGPGSSAAAAAGIYGSGPGVFGPYGSAAAAAGPGSGIYGIGPYGPGASGPGIYGPGVFGPSASAAAAAGSGVFGPGIYGPYASAAAAAGIYGSGPGVFGPYGPGISGSGVFGPGVFGPYASAAAAAGPGVFGPYGPGSSAAAAAGIYGYGPGVFGPYGPGASGINGPGSGIYGPGVFGPGISAAAAAGPGVFGPYGPGASAAAAAGIYGPGVFGPGIYGPGSSGPGVFGPYGPGSSAAAAAGIYGPGVFGPYGPGISAAAAAGIYVFGPGVFGPYGPGASGPGVFGPYGPGASAAAAAGPGIYGPGVFGPSASAAAAAGIYGSGPGIYGPYGPGISGPGSGVFGIGPYGPGASAAAAAGIYGPGVFGPYGPGISAAAAAGPGSGIYGPGASGINGPGSGIYGPGVFGPGISAAAAAGIYVFGPGVFGPYGPGASAAAAAGIYGSGPGVFGPYGPGISGSGVFGPGVFGPYASAAAAAGPGSGVFGPGAS